European Patent Application EP 4 549 591 A1, published May 7, 2025. Title: {A method of screening regulatory elements for enhancing mRNA translation, new regulatory elements according to the method, and use thereof. Applicant: Seoul National University R&DB Foundation. The sequence listing filed with the application follows.

SEQUENCE LISTING (187 sequences)

SEQ ID NO: 1 - DNA, 130 bp, Human gammaherpesvirus 4
  source 1..130: mol_type = genomic DNA
attaatgtccagtggggtaaatgcaccttgactgtaatcactggcaaagggcatgcttgggcatgctgtacctgatgagtcacaccccacggccatgctatcttgtaacggcatagggggaggggggaat

SEQ ID NO: 2 - DNA, 130 bp, Encephalomyocarditis virus
  source 1..130: mol_type = genomic DNA
cccccccccccccccccccccccccccccccccccccccccccccccccccccccccccccccccccctctccctcccccccccctaacgttactggccgaagccgcttggaataaggccggtgtgcgtt

SEQ ID NO: 3 - DNA, 130 bp, Human betaherpesvirus 5
  source 1..130: mol_type = genomic DNA
ggtcgctgacgtcaaaccatctcgtgctcgctgagtcacatccggttgttgacaagcgatggaggaccgcacccaaagtgcgccctctagtcatcgcgcctgaccccttttataaactgctcgaagaaaa

SEQ ID NO: 4 - DNA, 130 bp, Orf virus
  source 1..130: mol_type = genomic DNA
ccggaccccgcctgtgcgggcgagagcgcgctcgcgcagaacatcgacgtccagacgctagacctgggcgactgcggagaccccagaggccgccgactgcgcgtggcgctggtgaacagcggccacgcgg

SEQ ID NO: 5 - DNA, 130 bp, Molluscum contagiosum virus subtype 1
  source 1..130: mol_type = genomic DNA
ggcgagtcagtacatgcccggcctcgcctccgggcgcacaacttgggcccgcctccgggcagatagcaacctcgggaagccctcaggggctctcctacacattcctcggcgcacactcctcggcgctacg

SEQ ID NO: 6 - DNA, 130 bp, Borna disease virus 1
  source 1..130: mol_type = genomic DNA
ctggggtgaaaccgaggaggattcggtacaataagacctcacatgactaccacctggaggagtttgaggcaagtctcaacatgacccctcagaccagtatcgcctcgggtcatgagacagaccccataaa

SEQ ID NO: 7 - DNA, 130 bp, Husavirus sp.; identical to SEQ ID NO: 6
  source 1..130: mol_type = genomic DNA

SEQ ID NO: 8 - DNA, 130 bp, Human gammaherpesvirus 4
  source 1..130: mol_type = genomic DNA
gcttgggaacaccgggcaggtccgtgagaactttcttctactcgaggcctttttggcgtggtggcattaatgtccagtggggtaaatgcaccttgactgtaatcactggcaaagggcatgcttgggcatg

SEQ ID NO: 9 - DNA, 130 bp, Human herpesvirus 5
  source 1..130: mol_type = genomic DNA
tccattcctcgtaggctggtcctggggaacgggtcggcggccggtcggcttctgttttattattttttttttattttttatcttctcctttccttaatctcggattatcatttccctctcctacctacca

SEQ ID NO: 10 - DNA, 130 bp, Human herpesvirus 5
  source 1..130: mol_type = genomic DNA
caccgcgttatccattcctcgtaggctggtcctggggaacgggtcggcggccggtcggcttctgttttattattttttttttattttttatcttctcctttccttaatctcggattatcatttccctctc

SEQ ID NO: 11 - DNA, 130 bp, Saint Louis encephalitis virus
  source 1..130: mol_type = genomic DNA
agcatgctaaaggtgctgtctgtacatgccccaggaggactgggttaacaaagcttaacagccccagcggcccaaaccatggagtgcgtgaccatggcgtaaggactagaggttagaggagaccccgctg

SEQ ID NO: 12 - DNA, 130 bp, Breda virus
  source 1..130: mol_type = genomic DNA
tatgtctttttgttatggttaagtcatgttgttttagtggtcaaaaagttagatttaggtttagttaattcaggtggtgagagttatgtacttaggattttaagtagtgttaaggtgcccaattgtattg

SEQ ID NO: 13 - DNA, 130 bp, Human herpesvirus 5
  source 1..130: mol_type = genomic DNA
ctgccgtcgccaccgcgttatccattcctcgtaggctggtcctggggaacgggtcggcggccggtcggcttctgttttattattttttttttattttttatcttctcctttccttaatctcggattatca

SEQ ID NO: 14 - DNA, 130 bp, Human coronavirus OC43
  source 1..130: mol_type = genomic DNA
gctttagctaatatgttaccagcacatgtgtttatgaggttttatattattattgcctcttttattaagctctttagcttgtttaggcatgttgcctatggttgtagtaaatctggttgtttgttttgtt

SEQ ID NO: 15 - DNA, 130 bp, Sin Nombre orthohantavirus
  source 1..130: mol_type = genomic DNA
aagtctgttaaatgtagttaatcttgatagtattaagtcatatgtatggggggtgtttagtgttaagtcattgtttattgtttattgttatctgtttaatgctaagtctatatgatttattaatcaaaat

SEQ ID NO: 16 - DNA, 130 bp, Molluscum contagiosum virus subtype 1
  source 1..130: mol_type = genomic DNA
cgatggcgcgcgtgggctcggacttggccccttcgcttgtcgtgcttcctgcaaacttgacttgcggcgagtcagtacatgcccggcctcgcctccgggcgcacaacttgggcccgcctccgggcagata

SEQ ID NO: 17 - DNA, 130 bp, Human herpesvirus 5
  source 1..130: mol_type = genomic DNA
tatccgttcctcgtaggctggtcctggggaacgggtcggcggccggtcggcttctgttttatttttttttttattttttatcttctcctttccttaatctcggattatcatttccctctcctacctacca

SEQ ID NO: 18 - DNA, 130 bp, Human coronavirus HKU1
  source 1..130: mol_type = genomic DNA
tatgtaagcattttagtatgatgattttgagtgatgatggtgttgtctgttataactctgattatgctagtaagggttatatagctaatataagtgtttttcaacaagttttgtactatcagaataatgt

SEQ ID NO: 19 - DNA, 130 bp, Marburg marburgvirus
  source 1..130: mol_type = genomic DNA
agagagaacttcatttaattcacaaaaacaatctatttaagagtgagggttacattgtctaagatattgtatgagaagtaataaaataaataagaaaacgaaaagactattagacagcttattttataca

SEQ ID NO: 20 - DNA, 130 bp, Aichi virus 1
  source 1..130: mol_type = genomic DNA
catggttgtactgcactatcatcctaagacggtccttcttcggatcgcaatctcaccctggtgccgcgcttccttcgggaactgcacccgcggaccagggccgtctttgaacttttctaactgttcttac

SEQ ID NO: 21 - DNA, 130 bp, West Nile virus
  source 1..130: mol_type = genomic DNA
ccgaggtagaagaacaccgcaccgtccgtgtcctggagatggtggaagattggttgcacagaggaccgaaggaattctgcatcaaagtgctatgcccttacatgcccaaagtgattgagaagatggaaac

SEQ ID NO: 22 - DNA, 130 bp, Human coronavirus HKU1
  source 1..130: mol_type = genomic DNA
tattggttattcattatacacagtatggttttatccattattttgtcttattggtttacaattatttactacatggttgcctgatttgtttatgttagaaactatgcattggttgattagatttattgta

SEQ ID NO: 23 - DNA, 130 bp, Western chimpanzee simian foamy virus
  source 1..130: mol_type = genomic DNA
ctcagatgactagagatgaattagaagatactcttaatactcaaagtgaaatagaaattcaaatgataaatttattggaattgtatgaagtcgaaacaagggctctgcgaagacaactagcagaaagatc

SEQ ID NO: 24 - DNA, 130 bp, Bunyamwera virus
  source 1..130: mol_type = genomic DNA
ccagaggccctaggtataacaaaatggttcctgtctgtccagttgttttaagtgtcagggatgaattatttagaatgtctctagaaaatgtttttagtttaaacatgacaaactttagcatgtctagatt

SEQ ID NO: 25 - DNA, 130 bp, Molluscum contagiosum virus subtype 1
  source 1..130: mol_type = genomic DNA
acacacgcacccaaatcgcgtttgccaggcaacgcacaaaacacaaaaagaagtcgggcaaggcgtaagagcgtgaacatacgcactcgtggcaacaacatgaaggaaagtctttctcggccgccgtcac

SEQ ID NO: 26 - DNA, 130 bp, Human herpesvirus 5
  source 1..130: mol_type = genomic DNA
gactaccatcagcagtaccactaccgccacccccagcgccaccaccgctgccgtcgccaccgcgttatccgttcctcgtaggctggtcctggggaacgggtcggcggccggtcggcttctgttttatttt

SEQ ID NO: 27 - DNA, 130 bp, Cowpox virus
  source 1..130: mol_type = genomic DNA
ttatacatctggtggaggtggaatgtggggaggatcgtctagtggtgtaaaaagtggagttaatggaggtgttaacggaggtgtaaactctggagttaataaaatttaaacactaaattattttttatta

SEQ ID NO: 28 - DNA, 130 bp, Human herpesvirus 5
  source 1..130: mol_type = genomic DNA
ccactgccgccacccccagcgccaccaccgctgccgtcgccaccgcgttatccattcctcgtaggctggtcctggggaacgggtcggcggccggtcggcttctgttttattattttttttttatttttta

SEQ ID NO: 29 - DNA, 130 bp, Rotavirus A
  source 1..130: mol_type = genomic DNA
aaatcaattagcagtaaatggtataatgttgatgaattggataaattgccaatgtcaataaaatcaacggaggaactgattgaaatgaagaattctggaactttaactgaagaatttgagctactgatct

SEQ ID NO: 30 - DNA, 130 bp, Human herpesvirus 5
  source 1..130: mol_type = genomic DNA
gccaccaccgctgccgtcgccaccgcgttatccattcctcgtaggctggtcctggggaacgggtcggcggccggtcggcttctgttttattattttttttttattttttatcttctcctttccttaatct

SEQ ID NO: 31 - DNA, 130 bp, Breda virus
  source 1..130: mol_type = genomic DNA
gagttgattatttggatataagtgttttagatagttatgtaagtgataccgctggtttaaattgtgtacagaaggttaaaaagtttttatcaatgtattataattgtggtgctgatttgggtttgctaga

SEQ ID NO: 32 - DNA, 130 bp, Human coronavirus HKU1
  source 1..130: mol_type = genomic DNA
gtagataatgatttaaacccatttgttagcgatagtttagttacttattttggagattgtatgactttaccatttgattgtcattgggatttgataatatctgatatgtatgatcctcttactaaaaata

SEQ ID NO: 33 - DNA, 130 bp, Human coronavirus HKU1
  source 1..130: mol_type = genomic DNA
atactctaatgtttatcgtacagattatgttgattatacatttgttaatgagtattatgaatttttatgtaagcattttagtatgatgattttgagtgatgatggtgttgtctgttataactctgattat

SEQ ID NO: 34 - DNA, 130 bp, Human orthopneumovirus
  source 1..130: mol_type = genomic DNA
ctcaagaaactgattaaaataacaggtagtgtactatacaaccttcccaacgaacagtaacttaaaatatcattaacaagtttggtcaaatttagatgctaacacatcattatattatagttattaaaaa

SEQ ID NO: 35 - DNA, 130 bp, Variola virus
  source 1..130: mol_type = genomic DNA
tatcttcgaaaacaaaaatagatattatttttgcagtacaaactattgtttttatatggtttatattccactttgttcattcggcgatttaaaatttttattagttaaatggacatgatgcttatgattg

SEQ ID NO: 36 - DNA, 130 bp, Cowpox virus
  source 1..130: mol_type = genomic DNA
cagaatccgtcgtactgtttagttgtttaaaatttgttaatttactaatatctatatctttatcattattaatatctaaccatttatcattggtcttttttaaacttacccaataatctttataaaaaat

SEQ ID NO: 37 - DNA, 130 bp, Cowpox virus
  source 1..130: mol_type = genomic DNA
aaagtgagcaaaaattataaggttgtattctaatcccatatttgttatttttttctgtaatagttagaaaaatacattcgatggtctatctaccagattattatgtgttataaggtactttttctcataa

SEQ ID NO: 38 - DNA, 130 bp, Japanese encephalitis virus
  source 1..130: mol_type = genomic DNA
agggggtgcggcctgcgcagccccaggaggactgggttaccaaagccgttgagcccccacggcccaagcctcgtctaggatgcaatagacgaggtgtaaggactagaggttagaggagaccccgtggaaa

SEQ ID NO: 39 - DNA, 130 bp, Human herpesvirus 5
  source 1..130: mol_type = genomic DNA
atcagcagtaccactgccgccacccccagcgccaccaccgctgccgtcgccaccgcgttatccattcctcgtaggctggtcctggggaacgggtcggcggccggtcggcttctgttttattatttttttt

SEQ ID NO: 40 - DNA, 130 bp, NY_014 poxvirus
  source 1..130: mol_type = genomic DNA
atttacctaaaagtatgtataatgatatagtagagtttgttccagagaaactatatttatttaaatcacatattgtaaaaccactagatttgttatctatcttgatcaagttaaagaaagtggaaaaatt

SEQ ID NO: 41 - DNA, 130 bp, Hantaan orthohantavirus
  source 1..130: mol_type = genomic DNA
tatttctattgttctccttggttttactaagcattctctgtcccgtaaggaagcataaaaaatcatagctaaattctgtgactatcctgttcttatgtatagctttaacatatatactaatttttatatt

SEQ ID NO: 42 - DNA, 130 bp, Human coronavirus NL63
  source 1..130: mol_type = genomic DNA
gttagtaatgaatattgttgttttaaacatgcattgggttgtgattatgtttacaatccgtatgcttttgatatacaacagtggggttatgttggttccttgagccaaaaccaccacacattctgtaaca

SEQ ID NO: 43 - DNA, 130 bp, Severe acute respiratory syndrome coronavirus 2
  source 1..130: mol_type = genomic DNA
tattacggatgttttctacaaagaaaacagttacacaacaaccataaaaccagttacttataaattggatggtgttgtttgtacagaaattgaccctaagttggacaattattataagaaagacaattct

SEQ ID NO: 44 - DNA, 130 bp, NY_014 poxvirus
  source 1..130: mol_type = genomic DNA
ataataacctgtatcatttttctgacatcgttagtttcctcttgtatgttaaaatctattattttgaaatacgatgattctttccatagtgttacttacaaatgcatagatattaggacatgttatttgt

SEQ ID NO: 45 - DNA, 130 bp, Human coronavirus HKU1
  source 1..130: mol_type = genomic DNA
agattctaaacctcagcaagtcactaagcaaaatgccaaggaaatcaggcataaaattttaacaaaacctcgccaaaagcgaactcctaataaacattgtaatgttcaacagtgttttggtaaaagagga

SEQ ID NO: 46 - DNA, 130 bp, Human coronavirus HKU1
  source 1..130: mol_type = genomic DNA
ataaacgaaattgtagtgttcgtgttaagtgtagtactattgttggtggtgtaattcgttattatgatattactgctaatggtggtactggtttttgtgttaaacatcaatggaattgttttaattgcca

SEQ ID NO: 47 - DNA, 130 bp, Human coronavirus NL63
  source 1..130: mol_type = genomic DNA
taacaccagtcattgatgatgttgatgttgttaaaccttttagagttgaaggtaatttttcattctttgattgtggtgtcaatgccttggatggtgatatttacttattatttactaactctattttaat

SEQ ID NO: 48 - DNA, 130 bp, Human rhinovirus A1
  source 1..130: mol_type = genomic DNA
aataagaacactagttctagatgcatacaaaaatattgatctggacaagcttaaaataattgcatatggtgatgatgtgattttctcttataaatatactctagatatggaagctattgctaatgaagga

SEQ ID NO: 49 - DNA, 130 bp, Woodchuck hepatitis virus
  source 1..130: mol_type = genomic DNA
tccgggactttcgctttccccctccctattgccacggcggaactcattgccgcctgccttgcccgctgctggacaggggctcggctgttgggcactgacaattccgtggtgttgtcggggaagctgacgt

SEQ ID NO: 50 - DNA, 130 bp, Human coronavirus HKU1
  source 1..130: mol_type = genomic DNA
ttactacatggttgcctgatttgtttatgttagaaactatgcattggttgattagatttattgtatttgtagctaatatgttacctgcttttgtcttgttgcggttttatatagttgttactgctatgta

SEQ ID NO: 51 - DNA, 130 bp, Rubella virus
  source 1..130: mol_type = genomic DNA
ccgccgcgacagcgcgactccagcacctccggagatgactccggccgtgactccggagggccccgccgccgccgcggcaaccggggccgtggccagcgcagggactggtccagggccccgccccccccgg

SEQ ID NO: 52 - DNA, 130 bp, Rubella virus
  source 1..130: mol_type = genomic DNA
ccgccgccgcggcaaccggggccgtggccagcgcagggactggtccagggccccgccccccccggaggagcggcaagaaactcgctcccagactccggccccgaagccatcgcgggcgccgccacaacag

SEQ ID NO: 53 - DNA, 130 bp, Human herpesvirus 2
  source 1..130: mol_type = genomic DNA
gcgtcgtcgctgtcgtccgcctggggcaccagcagccagcgccgcaggagcgaggacgcggccggcgcgctctcgaccgcggttcccgagtcgtacgcagggaccatttgggagtctgcggttgggagcg

SEQ ID NO: 54 - DNA, 130 bp, Yellow fever virus
  source 1..130: mol_type = genomic DNA
agagagaagaagctgtcagagtttgggaaagcaaagggaagccgtgccatatggtatatgtggctgggagcgcggtatcttgagtttgaggccctgggattcctgaatgaggaccattgggcttccaggg

SEQ ID NO: 55 - DNA, 130 bp, Human gammaherpesvirus 8
  source 1..130: mol_type = genomic DNA
gaggatcacccagccttttgcgatgtgccggtcacgcagacgggcgcggaatctgaggactctggagacgagggaccatcgacgcgccatagtgcgtctggggttcagccagttgatgatgccaatgccg

SEQ ID NO: 56 - DNA, 130 bp, Saint Louis encephalitis virus
  source 1..130: mol_type = genomic DNA
acgacgtgaattgaaatgtggaggaggcatcttcgtgtacaacgacgttgagaagtggaagagcgactacaagtatttccctctgactccaactggactcgcgcgtgtgattcaagaggcgcatgccaat

SEQ ID NO: 57 - DNA, 130 bp, NY_014 poxvirus
  source 1..130: mol_type = genomic DNA
gacataatagtttttggtttgttattattagatcaattgctggtatgataatgtacttggtacttggtataatactgttatatatttcagagaagaagaatgataatgatatttcaaaggaaagtacttc

SEQ ID NO: 58 - DNA, 130 bp, GB virus C
  source 1..130: mol_type = genomic DNA
ctcgatgagcgcaggggggtggaggcacaaagccgtgatctataggacgtggtgtaaggggtaccaggcaatccgtcaaagggtggtgaggagccccctcggggaggggcggcctgccaaacccctgacc

SEQ ID NO: 59 - DNA, 130 bp, Middle East respiratory syndrome-related coronavirus
  source 1..130: mol_type = genomic DNA
aaaatcccagtgttattggtgtttatcataaacttggagaacgtgtacgccaagctatcttaaacactgttaaattttgtgaccacatggtcaaggctggtttagtcggtgtgctcacactagacaacca

SEQ ID NO: 60 - DNA, 130 bp, Mammalian orthoreovirus 3
  source 1..130: mol_type = genomic DNA
gagagatgatgctggtcaacaagtttgccccgactatgtcatgcttcggtcctctgtcacgacaaaagtggtgcggaatgtggttgagtaccagatccgtacgggtggattcttttcgtgcttagctatg

SEQ ID NO: 61 - DNA, 130 bp, Human herpesvirus 5
  source 1..130: mol_type = genomic DNA
gcaagatgggcaccgtctgttcgcaaggtaagccccacgtcgttgaagacacctggaaagaggacgttcgctcgggcacgttctttccaggtgttttcaacgtgcgtggattttttctattctctaccag

SEQ ID NO: 62 - DNA, 130 bp, Molluscum contagiosum virus subtype 1
  source 1..130: mol_type = genomic DNA
tggccttgcgagcgctgcctgtgctacgcgagcactgcgcgcgcggcgcagtgctctttagtacaacgcgctacgtactctccaactatttcaacccctcggaggaaaagcacgcggccatttacttcgg

SEQ ID NO: 63 - DNA, 130 bp, Infectious spleen and kidney necrosis virus
  source 1..130: mol_type = genomic DNA
accgcgtcgtgtccatgctgggcttcgacaaggaccccaaggtcggagcacggatggtcgacgtcatcatgtccatgctgagcaccccgcgtgacgccacaaggccacgtacgccacgcggctgggccgt

SEQ ID NO: 64 - DNA, 130 bp, Dengue virus 1
  source 1..130: mol_type = genomic DNA
gcagcggggcccaacaccaggggaagctgtaccctggtggtaaggactagaggttagaggagaccccccgcacaacaacaaacagcatattgacgctgggagagaccagagatcctgctgtctctacagc

SEQ ID NO: 65 - DNA, 130 bp, Human astrovirus
  source 1..130: mol_type = genomic DNA
tttatggagatgacaggctttctacaacaccttcggtgcccgatgattatgaggagagagtgatcactatgtatagagacatctttggcatgtgggttaagcctgggaaggttatctgtagagacagcat

SEQ ID NO: 66 - DNA, 130 bp, Norovirus GII
  source 1..130: mol_type = genomic DNA
gtgtactcaaatcaaactatttcaacgagacttggttctacagctggttctggaaccagtgtctcgagcctcccgtcaactgcaaggactaggagctgggttgaggaccaaagtaggaatctgtcacctt

SEQ ID NO: 67 - DNA, 130 bp, Severe acute respiratory syndrome coronavirus 2
  source 1..130: mol_type = genomic DNA
ttggtatgcaaaagtattctacactccagggaccacctggtactggtaagagtcattttgctattggcctagctctctactacccttctgctcgcatagtgtatacagcttgctctcatgccgctgttga

SEQ ID NO: 68 - DNA, 130 bp, Saint Louis encephalitis virus
  source 1..130: mol_type = genomic DNA
gcatggtgttcactcgattgtggctcacaatccgggaggaaaacacaacggaatgcgattcggcaatcatcggcacagctataaaaggagacagagctgttcacagtgacctatcgtattggattgagag

SEQ ID NO: 69 - DNA, 130 bp, Human astrovirus
  source 1..130: mol_type = genomic DNA
tgaacaactacctgagttacttttacagggcgtctgccactggggatgccacaactaacctgttggttagaggagacacatacacagcagggataagttttacccagggtggatggtatttgttgacaaa

SEQ ID NO: 70 - DNA, 130 bp, Human immunodeficiency virus 1
  source 1..130: mol_type = genomic DNA
ctttccatccctgtggaagcacattgtactgatatctaatccctggtgtctcattgtttatactaggtatggtaaatgcagtatacttcctgaagtcttcatctaagggaactgaaaaatatgcatcacc

SEQ ID NO: 71 - DNA, 130 bp, Molluscum contagiosum virus subtype 1
  source 1..130: mol_type = genomic DNA
gaggggaaagatgaagctctcgcgcgcagggcgcgaacctagacacgagcgcggcaacagcacgacgaagaaggttctggtgtccgcagtaccggccaaggcaaagttctcgcgttcgcgttcgacagct

SEQ ID NO: 72 - DNA, 130 bp, Human coronavirus HKU1
  source 1..130: mol_type = genomic DNA
tagtcagggtaaagactttggttatgtatgtgatggttctttttataaagcaactgttaatcaagtttgtgttttattagctaagaagatagatgttttgcttactgtagatggtgttaattttaaatct

SEQ ID NO: 73 - DNA, 130 bp, Great Island virus
  source 1..130: mol_type = genomic DNA
acgttacgctacagatgtgtacgctgagggtgatgtatcatggcttacaatcaggcaggtgcgtgcacacggcatcatcttcgtgggacccgcaggggcacggttcccgatgcgcgatgcagttctttca

SEQ ID NO: 74 - DNA, 130 bp, Great Island virus
  source 1..130: mol_type = genomic DNA
cccgatgtgataatacggagcgtcagagacgcgaaagatttggagacgcagattggacgcggacgcataaaactaaggcgtaccttcgggaacgcggttcgtaactacgcatgggcgcgagcgacctatt

SEQ ID NO: 75 - DNA, 130 bp, Influenza C virus
  source 1..130: mol_type = genomic DNA
gactgatatcaaactgaatttccagaaaaacatttatgaactggcttcacaatcacattgcatgagcttggtgaatgccttggacaaaactattcctttacaagcgactgcaggggttgcaaaaaattgc

SEQ ID NO: 76 - DNA, 130 bp, Human betaherpesvirus 5
  source 1..130: mol_type = genomic DNA
tcatgatttctacgggtatctgcagctggaccttctgggaccagtggtggcggggaatcgctcagtccggacctggagagagcaggcggaccgagccagagggaccttcgttcggcgttcaggccttaat

SEQ ID NO: 77 - DNA, 130 bp, Astrovirus MLB1
  source 1..130: mol_type = genomic DNA
aaaggggtcctcggaggaggaccccaaacactacctagatacatggattgggatgcttagtccttgcgttcgttggctggttccggaacgctttcctttgtatggtggtgtacctttagataggccagtg

SEQ ID NO: 78 - DNA, 130 bp, Severe fever with thrombocytopenia syndrome virus
  source 1..130: mol_type = genomic DNA
ctcatccaaggattttgtgtgctataaggaagggactgggccgtgttctgaatcagaagaaaagacttgcaagaccagtggatcatgcaggggggacatgcagttttgcaaggtggcaggttgtgaacat

SEQ ID NO: 79 - DNA, 130 bp, Sin Nombre orthohantavirus
  source 1..130: mol_type = genomic DNA
cacagggtatataatctatattgtttagtgttattgtagtattgtattatgtattgttagttaagcttattaaatcttgttaagtttgttaagttttgttaagttgtattaagttttgttaagtttcggt

SEQ ID NO: 80 - DNA, 130 bp, Sin Nombre orthohantavirus; identical to SEQ ID NO: 15
  source 1..130: mol_type = genomic DNA

SEQ ID NO: 81 - DNA, 130 bp, Norovirus GII
  source 1..130: mol_type = genomic DNA
ttagggatgctgtccctgctcggggaccctccaataaatcttctaactcttctactgccacctctgtgtactcaaatcaaactatttcaacgagacttggttctacagctggttctggaaccagtgtctc

SEQ ID NO: 82 - DNA, 130 bp, Saffold virus
  source 1..130: mol_type = genomic DNA
aacatcctctcgatcggatcgcaacgtgttacccaggaatccacttgggtgtacgcggccgttctgacgttggaattctgtagatgaaagttagctaggagcttttaattggaaatgagaacaaaaaaaa

SEQ ID NO: 83 - DNA, 130 bp, Vesicular exanthema of swine virus
  source 1..130: mol_type = genomic DNA
ttttatcagtttattatcttagttacttaagtgttttatactttcacctctgtgtatctatataatcaatgggataattgttcttaatctagtagactgtagaattagttaattggtaggttgcattagg

SEQ ID NO: 84 - DNA, 130 bp, Japanese encephalitis virus; identical to SEQ ID NO: 38
  source 1..130: mol_type = genomic DNA

SEQ ID NO: 85 - DNA, 130 bp, Tick-borne encephalitis virus
  source 1..130: mol_type = genomic DNA
ctccgctgtggcgagggcctggtcgtgtggagagaggtctcagaatggtatgacaattatgcctactacccggagacaccgggggcccttgcatcagccataaaggagacatttgaggagggaagctgtg

SEQ ID NO: 86 - DNA, 130 bp, Human coronavirus 229E
  source 1..130: mol_type = genomic DNA
gtaacaatgattgcttatgccatattgtatttctttgctactagaagcttacgctatgcatggatttggtgtgctgcatatttaattgcgtatatttcttttgctccatggtggttgtgtgcttggtact

SEQ ID NO: 87 - DNA, 130 bp, Human coronavirus NL63
  source 1..130: mol_type = genomic DNA
attctgttttcacttgttttcaaataagtaaggactcaaaattccaaataggtgagttcatctttgagaaggttgaatatggttctgatactgttacgtataagtctactgtaactactaagttagttcc

SEQ ID NO: 88 - DNA, 130 bp, Breda virus
  source 1..130: mol_type = genomic DNA
tagctgtctcaagtttagggtttattaaccctcttatgtggcccctgtttattgttgttttgcttgataataggtttgtttggttttttaatgtgttaagttatatcatgttaccagtttttgtgattat

SEQ ID NO: 89 - DNA, 130 bp, SARS coronavirus Tor2
  source 1..130: mol_type = genomic DNA
ctgctcaattaccagccccccgcacattgctgactaaaggcacactagaaccagaatattttaattcagtgtgcagacttatgaaaacaataggtccagacatgttccttggaacttgtcgccgttgtcc

SEQ ID NO: 90 - DNA, 130 bp, Human coronavirus HKU1
  source 1..130: mol_type = genomic DNA
tatctaattcagagtggtattttctttacatctttgatgtctcaattttcacaagaagtttctgatatgtgtttaaaaatgtgtattttgtttatggacagagtttcagttgctacattttatatagagc

SEQ ID NO: 91 - DNA, 130 bp, Human coronavirus HKU1
  source 1..130: mol_type = genomic DNA
agttttattttgtcttatttctttaatctttgttgttgcttttttagcaactattaagctttgtatgcaactttgtggtttttgtaatttctttattatttcaccttcggcttacgtttataaaagaggt

SEQ ID NO: 92 - DNA, 130 bp, Human coronavirus OC43
  source 1..130: mol_type = genomic DNA
taatatccctgatttacccatttgtgtgtatgatccgctaccagttattttgcttggcattcttttgggcgttgcgattgtaattattgtagttttgttgttatattttatggtggataatgttactagg

SEQ ID NO: 93 - DNA, 130 bp, NY_014 poxvirus
  source 1..130: mol_type = genomic DNA
ttttcttaacttttaaaatgtctaggttttgttttgttaacaatgacaaatggttttttattaaccactcaaaaaagtaatttgatatttcatatcctctattggctgttatttcattaccatgtataaa

SEQ ID NO: 94 - DNA, 185 bp, Aichi virus 1
  source 1..185: mol_type = genomic DNA
cactcctccatggtgatataaagaccacccacttccttcgggtgagcccctaagccatggttgtactgcactatcatcctaagacggtccttcttcggatcgcaatctcaccctggtgccgcgcttccttcgggaactgcacccgcggaccagggccgtctttgaacttttctaactgttcttac

SEQ ID NO: 95 - DNA, 120 bp, Aichi virus 1
  source 1..120: mol_type = genomic DNA
ctgcactatcatcctaagacggtccttcttcggatcgcaatctcaccctggtgccgcgcttccttcgggaactgcacccgcggaccagggccgtctttgaacttttctaactgttcttac

SEQ ID NO: 96 - DNA, 20 bp, synthetic construct
  source 1..20: mol_type = other DNA
acctcaggacggacttaccg

SEQ ID NO: 97 - DNA, 22 bp, synthetic construct
  source 1..22: mol_type = other DNA
caagtgggcagcgcgcgccgcc

SEQ ID NO: 98 - DNA, 130 bp, Canine kobuvirus US-PC0082
  source 1..130: mol_type = genomic DNA
taagccatggttgtactgtgctatctttctaagacgtcctctctttggacgcactttccccctggcgccgcgcctccctcgggagctgcacccgcgggccagggttgtctttgaacttttctaactgttc

SEQ ID NO: 99 - DNA, 130 bp, Canine kobuvirus
  source 1..130: mol_type = genomic DNA
catggttgtactgtgctatctttctaagacgtcctctctctggacgcactttccccctggcgccgcgcctccctcgggagctgcacccgcgggccagggttgtctttgaacttttctaactgttcttaaa

SEQ ID NO: 100 - DNA, 130 bp, Kobuvirus sp.
  source 1..130: mol_type = genomic DNA
ccatggttgtactgcactatcaatctaagacggtccttcttcggatcgcatttccccctggtgccgcgcctcccccgggagctgcacccgcggaccagggcagtctttgaacttttctaactgttcttac

SEQ ID NO: 101 - DNA, 130 bp, Kobuvirus sewage Aichi
  source 1..130: mol_type = genomic DNA
agccatggttgtactgtgctatctttctaagacgtcctctctctggacgcactttccccctggcgccgcgcttccctcgggaactgcacccgcgggccagggttgtctttgaacttttctaactgttctt

SEQ ID NO: 102 - DNA, 130 bp, Feline kobuvirus
  source 1..130: mol_type = genomic DNA
catggttgtactgctctatctcctaagacgtcctctctctggacgcactttcaccctggtgccgcgcctcttcggagctgcacccgcggaccagggtagtctttgaacttttctaactgttcttaaaaaa

SEQ ID NO: 103 - DNA, 130 bp, Aichivirus A
  source 1..130: mol_type = genomic DNA
catggttgtactgtgctatctctctaagacggtctctctctgaccgcatttcccccctggcgccgcgctccttcgggactgcacccgcgggccagggttgtctttgagcttttctaactgttcttataaa

SEQ ID NO: 104 - DNA, 130 bp, Kobuvirus SZAL6-KoV/2011/HUN
  source 1..130: mol_type = genomic DNA
ttgctagaaagaaacctttatactatccctaagaccaggctctttcctggcaatttcaccgggtagccgcgctccgaaaggactgcacccgcggtacccggtacgtctttgaacttttctttctgttctt

SEQ ID NO: 105 - DNA, 130 bp, Canine kobuvirus CH-1
  source 1..130: mol_type = genomic DNA
catggttgtactgtgctatctttctaagacgtcctctctctggacgcactttccccctggcgccgcgcctccctcgggaactgcacccgcgggccagggttgtctttgaacttttctaactgttcttaaa

SEQ ID NO: 106 - DNA, 130 bp, Kobuvirus sp.
  source 1..130: mol_type = genomic DNA
gagcccctaagccttggtcgtactgcactatctctctaagacggtctctctctgaccgcactttccccccagcgccgcgctccctcgggactgcacccgcgggctggggttgtctttgaacttttctaac

SEQ ID NO: 107 - DNA, 130 bp, Aichivirus A
  source 1..130: mol_type = genomic DNA
agccatagttgtactgcactatctttctaagacggtctctctctgaccgcactttccccctggcgccgcgctccttcgggactgcacccgcgggccagggtagtctttgagcttttctaactgttcttat

SEQ ID NO: 108 - DNA, 130 bp, Mouse kobuvirus M-5/USA/2010
  source 1..130: mol_type = genomic DNA
catggttgtactgtgctatcttctaagacgtcctccctctggacgcactttccccccggtgccgcgcctcccctgggagctgcacccgcggaccggggtagtctttgaacttttctaactgttcttaaaa

SEQ ID NO: 109 - DNA, 130 bp, Canine kobuvirus
  source 1..130: mol_type = genomic DNA
catggttgtactgtgctatctttctaagacgtcctctctctggacgcactttctccctggtgccgcgcttccttcgggaactgcacccgcggaccagggtcgtctttgagcttttctaactgtttttaaa

SEQ ID NO: 110 - DNA, 130 bp, Feline kobuvirus
  source 1..130: mol_type = genomic DNA
catggttgtactgctctatcttctaagacgtcctctctctggacgcactttcaccctggtgccgcgcctcttctgagctgcacccgcggaccagggtagtctttgaacttttctagctgttcttaaaaaa

SEQ ID NO: 111 - DNA, 130 bp, Kobuvirus sewage Kathmandu
  source 1..130: mol_type = genomic DNA
cttggtcgtactgcactatctctctaagacggtctctctttgaccgcactttccccccagcgccgcgctccttcgggactgcacccgcgggctggggttgtctttgaacttttctaactgttcttgaaaa

SEQ ID NO: 112 - DNA, 130 bp, Feline kobuvirus
  source 1..130: mol_type = genomic DNA
catggttgtactgctctatcttctaagacgtcctctctctggacgcactttcaccctggtgccgcgcctctcttgagctgcacccgcggatcagggtagtctttgaacttttctacctgttcttacaaaa

SEQ ID NO: 113 - DNA, 130 bp, Aichi virus 1
  source 1..130: mol_type = genomic DNA
catggttgtactgcactatcaatctaagacggtccttcttcgggccgcactttccccctggtgccgcgcctcccccgggagctgcacccgcggaccagggttgtctttgaacttttctaactgttcttat

SEQ ID NO: 114 - DNA, 130 bp, Canine kobuvirus
  source 1..130: mol_type = genomic DNA
catggtcgtactgtgctatctttctaagacgtcctctctctggacgcactttctccctggtgccgcgcttccctcgggaactgcacccgcggaccagggtcgtctttgaacttttctaactgttcttaaa

SEQ ID NO: 115 - DNA, 130 bp, Kobuvirus dog/AN211D/USA/2009
  source 1..130: mol_type = genomic DNA
catggttgtactgtgctatctttctaagacgtcctctctttggacgcactttccccctggcgccgcgcctccctcgggaactgcacccgcgggccagggttgtctttgaacttttctaactgttcttaaa

SEQ ID NO: 116 - DNA, 130 bp, Aichivirus A
  source 1..130: mol_type = genomic DNA
catggttgtactgcactatcaatctaagacggtccttcttcggatcgcattttccccctggtgccgcgcctcccccgggagctgcacccgcggaccagggtagtctttgaacttttctaactgttcttac

SEQ ID NO: 117 - DNA, 130 bp, Kobuvirus sp.
  source 1..130: mol_type = genomic DNA
cttggtcgtactgcactatctctctaagacggtctctctctgaccgcactttccccccagcgccgcgctccctcgggactgcacccgcgggctggggttgtctttgaacttttctaactgttcttgaaaa

SEQ ID NO: 118 - DNA, 130 bp, Aichivirus A7
  source 1..130: mol_type = genomic DNA
gtgattagaatcctttatgctgtccctaagaccaggctctcccctggcactttcccccggttgccgcgccctctctgaggctgcacccgcggaaccgggttgtccttgaacttttctaatcgttcttgca

SEQ ID NO: 119 - DNA, 130 bp, Feline kobuvirus
  source 1..130: mol_type = genomic DNA
catggttgtactgctctatctcctaagacgtcctctctctggacgcactttcaccctggtgccgcgcctctcctgagctgcacccgcggatcagggtagtctttgaacttttctagctgttcttaaaaaa

SEQ ID NO: 120 - DNA, 130 bp, Canine kobuvirus
  source 1..130: mol_type = genomic DNA
catggtcgtactgtgctatctttccaagacgtcctctctctggacgcactttctccctggtgccgcgcttccctcgggaactgcacccgcggaccagggtcgtctttgaacttttctaactgttcttaaa

SEQ ID NO: 121 - DNA, 130 bp, Feline kobuvirus
  source 1..130: mol_type = genomic DNA
catggttgtactgctctatcttctaagacgtcctctctctggacgcactttcaccctggtgccgcgcctcttctgagctgcacccgcggaccagggtagtctttgaacttttctagctgttcttacaaaa

SEQ ID NO: 122 - DNA, 130 bp, Aichi virus 1
  source 1..130: mol_type = genomic DNA
catggttgtactgcactatcaacctaagacggtccttctccggatcgcactttccccctggtgccgcgcctcccgcgggagctgcacccgcggaccagggtagtctttgaacttttctaactgttcttac

SEQ ID NO: 123 - DNA, 130 bp, Aichi virus 1
  source 1..130: mol_type = genomic DNA
ccatggttgtactgcactatcaatctaagacggtccttcttcggatcgcatttccccctggtgtcgcgcctcccccgggagctgcacccgcggaccagggtagtctttgaacttttctaactgttcttac

SEQ ID NO: 124 - DNA, 130 bp, Aichi virus 1
  source 1..130: mol_type = genomic DNA
catggttgtactgcactatcaatctaagacggtccttctccggatcgcactttcctcctggtgccgcgcctccttcgggagctgcacccgcggaccaggatagtctttgaacttttctaactgttcttac

SEQ ID NO: 125 - DNA, 130 bp, Aichi virus 1
  source 1..130: mol_type = genomic DNA
catggttgtactgcactatcaacctaagacggtccttctccgggtcgcactttccccctggtgccgcgcctcccgcgggagctgcacccgcggaccagggtagtctttgaacttttctaactgttcttac

SEQ ID NO: 126 - DNA, 130 bp, Canine kobuvirus 1
  source 1..130: mol_type = genomic DNA
catggtcgtactgtgctatctttccaagacgtcctctctctggacgcactttctccctggtgccgcgcttccctcgggaactgcacccgcggaccaggattgtctttgaacttttctaactgttcttaaa

SEQ ID NO: 127 - DNA, 130 bp, Aichi virus 1
  source 1..130: mol_type = genomic DNA
catggttgtactgcactatcaatctaagacggtccttcttcggatcgcaatttcactctggtgccgcgcttcctccgggaactgcacccgcggaccagggtcgtctttgaacttttctaactgtttctta

SEQ ID NO: 128 - DNA, 130 bp, Canine kobuvirus 1
  source 1..130: mol_type = genomic DNA
catggtcgtactgtgctatctttccaagacgtcctctctctggacgcactttctccctggtgccgcgcttccctcgggaactgcacccgcggaccagggtcgtctttgaactcttctaactgttcttaaa

SEQ ID NO: 129 - DNA, 130 bp, Aichi virus 1
  source 1..130: mol_type = genomic DNA
catggttgtactgcactatcaatctaagacggtccttcttcggatcgcaatttcactccggtgccgcgcttcctccaggaactgcacccgcggaccggggtcgtctttgaacttttctaactgttcttac

SEQ ID NO: 130 - DNA, 130 bp, Aichi virus 1
  source 1..130: mol_type = genomic DNA
cgtggttgtattgcactatcaatctaagacggtcctccttcggatcgcaatttcaccctggtgtcgcgcttcctccgggaactgcacccgcggaccagggtcgtctttgaacttttctaactgttcttat

SEQ ID NO: 131 - DNA, 130 bp, Canine kobuvirus
  source 1..130: mol_type = genomic DNA
cgggtgagcccctaagccatggttgtactgtgctatctttctaagacgccctctctctggacgcactttctccctggtgccgcgcttccttcgggaactgcacccgcggaccagggccgtctttgaactt

SEQ ID NO: 132 - DNA, 130 bp, Canine kobuvirus 1
  source 1..130: mol_type = genomic DNA
catggtcgtactgtgctatctttccaagacgtcctctctctggacgcactttctccctggtgccgcgcttccctcgggaactgcacccgcggaccaggatcgtctttgaactcttctaactgttcttaaa

SEQ ID NO: 133 - DNA, 130 bp, Canine kobuvirus 1
  source 1..130: mol_type = genomic DNA
catggttgtactgtgctgtctttctaagacgtcctctctctggacgcacttcctccctggtgccgcgcttcccccgggaactacacccgcggaccagggccgtctttgaacttttctaactgttcttaaa

SEQ ID NO: 134 - DNA, 130 bp, Feline kobuvirus
  source 1..130: mol_type = genomic DNA
agttagttagaaccctctgctctcctccatgatgatataaagaccacccattacttttcgggtgagcccctaagtcatggttgtactgctctatcttctaagacgtcctctctctggacgcactttcacc

SEQ ID NO: 135 - DNA, 130 bp, Marmot kobuvirus
  source 1..130: mol_type = genomic DNA
gagtgagcccctaagctgtggttgtactgcactatcttctaagacgccctctctttgggcgcacctccccccggtgccgcgctccctcgcgggactgcacccgcggaccggggtagtctttgaacttttc

SEQ ID NO: 136 - DNA, 130 bp, Canine kobuvirus
  source 1..130: mol_type = genomic DNA
accccttcactcctccatggtgatataaagaccacccacaaacttttcgggtgagcccctaagccatggttgtactgtgctatctttctaagacgtcttctctctagacgcactttccccctggcgccgc

SEQ ID NO: 137 - DNA, 130 bp, Canine kobuvirus
  source 1..130: mol_type = genomic DNA
accccttcactcctccatggtgatataaagaccacccacaaacttttcgggtgagcccctaagccatggttgtactgtgctatctttctaagacgtcctctctctggacgcactttccccctggcgccgc

SEQ ID NO: 138 - DNA, 130 bp, Canine kobuvirus
  source 1..130: mol_type = genomic DNA
accccttcactcctccatggtgatataaagaccacccacaaacttttcgggtgagcccctaagccatggttgtactgtgctatctctctaagacgtcctctctctggacgcactttccccctggcgccgc

SEQ ID NO: 139 - DNA, 130 bp, Murine kobuvirus
  source 1..130: mol_type = genomic DNA
gccatagtcgtactggactatctttaagacggcactttttcgtgtcgcactttccccccggcgccgcgcctcctccgggagctgcacccgcgggccggggtcgtctttgaacttttctagttgttcttac

SEQ ID NO: 140 - DNA, 130 bp, Canine kobuvirus
  source 1..130: mol_type = genomic DNA
catggttgtactgtgctatctttctaagacgtctcctctctggacgcactttccccttggcgccgccgccctccctcggggagctgcaccccgcgggccagggttgtctttgaacttttctaactgttct

SEQ ID NO: 141 - DNA, 20 bp, synthetic construct
  source 1..20: mol_type = other DNA
cccatcttcggcaaccagat

SEQ ID NO: 142 - DNA, 20 bp, synthetic construct
  source 1..20: mol_type = other DNA
gtacatgagcacgacccgaa

SEQ ID NO: 143 - DNA, 19 bp, synthetic construct
  source 1..19: mol_type = other DNA
ctggacgaagagcatcagg

SEQ ID NO: 144 - DNA, 20 bp, synthetic construct
  source 1..20: mol_type = other DNA
tgatattcggcaagcaggca

SEQ ID NO: 145 - DNA, 20 bp, synthetic construct
  source 1..20: mol_type = other DNA
aagcagaagaacggcatcaa

SEQ ID NO: 146 - DNA, 20 bp, synthetic construct
  source 1..20: mol_type = other DNA
gggggtgttctgctggtagt

SEQ ID NO: 147 - DNA, 22 bp, synthetic construct
  source 1..22: mol_type = other DNA
gtaactacgccctgaccttgct

SEQ ID NO: 148 - DNA, 22 bp, synthetic construct
  source 1..22: mol_type = other DNA
agccatcgacttccacctgttc

SEQ ID NO: 149 - DNA, 22 bp, synthetic construct
  source 1..22: mol_type = other DNA
agttcgtccgttagtgctggtg

SEQ ID NO: 150 - DNA, 22 bp, synthetic construct
  source 1..22: mol_type = other DNA
gagggatggaaggatgggttca

SEQ ID NO: 151 - DNA, 22 bp, synthetic construct
  source 1..22: mol_type = other DNA
aggcaccaagagaaacgccgat

SEQ ID NO: 152 - DNA, 23 bp, synthetic construct
  source 1..23: mol_type = other DNA
catagaaccgcagcaattccacc

SEQ ID NO: 153 - DNA, 20 bp, synthetic construct
  source 1..20: mol_type = other DNA
cccaccacttccagaacact

SEQ ID NO: 154 - DNA, 20 bp, synthetic construct
  source 1..20: mol_type = other DNA
gctttcaaagacgcagttcc

SEQ ID NO: 155 - DNA, 17 bp, synthetic construct
  source 1..17: mol_type = other DNA
tcgcagatgaggattcg

SEQ ID NO: 156 - DNA, 18 bp, synthetic construct
  source 1..18: mol_type = other DNA
ctgctctcacgccattct

SEQ ID NO: 157 - DNA, 23 bp, synthetic construct
  source 1..23: mol_type = other DNA
ccttgaacagcagaggaagttgg

SEQ ID NO: 158 - DNA, 22 bp, synthetic construct
  source 1..22: mol_type = other DNA
ggagatgaggttcagagtctgc

SEQ ID NO: 159 - DNA, 22 bp, synthetic construct
  source 1..22: mol_type = other DNA
ctctctgctcctcctgttcgac

SEQ ID NO: 160 - DNA, 19 bp, synthetic construct
  source 1..19: mol_type = other DNA
tgagcgatgtggctcggct

SEQ ID NO: 161 - DNA, 21 bp, synthetic construct
  source 1..21: mol_type = other DNA
ccatgatcacgaaggtggttt

SEQ ID NO: 162 - DNA, 21 bp, synthetic construct
  source 1..21: mol_type = other DNA
atgcagtcgagtttcccacat

SEQ ID NO: 163 - DNA, 20 bp, synthetic construct
  source 1..20: mol_type = other DNA
gtaacccgttgaaccccatt

SEQ ID NO: 164 - DNA, 20 bp, synthetic construct
  source 1..20: mol_type = other DNA
ccatccaatcggtagtagcg

SEQ ID NO: 165 - DNA, 22 bp, synthetic construct
  source 1..22: mol_type = other DNA
gcacccggctttctccttccac

SEQ ID NO: 166 - DNA, 22 bp, synthetic construct
  source 1..22: mol_type = other DNA
tgcacggctctacctccacctc

SEQ ID NO: 167 - DNA, 22 bp, synthetic construct
  source 1..22: mol_type = other DNA
aaggcccaaactgcactgcaca

SEQ ID NO: 168 - DNA, 22 bp, synthetic construct
  source 1..22: mol_type = other DNA
cacttggggttgctgcaggtgt

SEQ ID NO: 169 - DNA, 31 bp, synthetic construct
  source 1..31: mol_type = other DNA
tgataagcagagctcactggccgcttcactg

SEQ ID NO: 170 - DNA, 33 bp, synthetic construct
  source 1..33: mol_type = other DNA
tcgtgcttgcggccgccgacgctcttccgatct

SEQ ID NO: 171 - DNA, 45 bp, synthetic construct
  source 1..45: mol_type = other DNA
gttcagagttctacagtccgacgatcnncgacgctcttccgatct

SEQ ID NO: 172 - DNA, 46 bp, synthetic construct
  source 1..46: mol_type = other DNA
gttcagagttctacagtccgacgatcnnncgacgctcttccgatct

SEQ ID NO: 173 - DNA, 44 bp, synthetic construct
  source 1..44: mol_type = other DNA
gttcagagttctacagtccgacgatcncgacgctcttccgatct

SEQ ID NO: 174 - DNA, 44 bp, synthetic construct
  source 1..44: mol_type = other DNA
gccttggcacccgagaattccanngcaagatcgccgtgtaattc

SEQ ID NO: 175 - DNA, 45 bp, synthetic construct
  source 1..45: mol_type = other DNA
gccttggcacccgagaattccannngcaagatcgccgtgtaattc

SEQ ID NO: 176 - DNA, 43 bp, synthetic construct
  source 1..43: mol_type = other DNA
gccttggcacccgagaattccangcaagatcgccgtgtaattc

SEQ ID NO: 177 - DNA, 48 bp, synthetic construct
  source 1..48: mol_type = other DNA
taatacgactcactatagggagagggcctttcgacctgcagcccaagc

SEQ ID NO: 178 - DNA, 143 bp, synthetic construct
  misc_feature 1..2: note = 2'-O-Methylated deoxyuridine
  source 1..143: mol_type = other DNA
ttttttttttttttttttttttttttttttttttttttttttttttttttttttttttttttttttttttttttttttttttttttttttttttttttttttttttttttttttttttttatcaatgtatcttatcatgtctg

SEQ ID NO: 179 - DNA, 46 bp, synthetic construct
  source 1..46: mol_type = other DNA
taatacgactcactatagggagagggaaataagagagaaaagaaga

SEQ ID NO: 180 - DNA, 21 bp, synthetic construct
  source 1..21: mol_type = other DNA
ggacaaaccacaactagaatg

SEQ ID NO: 181 - DNA, 47 bp, synthetic construct
  source 1..47: mol_type = other DNA
gttcagagttctacagtccgacgatcggacaaaccacaactagaatg

SEQ ID NO: 182 - DNA, 20 bp, synthetic construct
  source 1..20: mol_type = other DNA
acctcaggacggacttaccg

SEQ ID NO: 183 - DNA, 19 bp, synthetic construct
  source 1..19: mol_type = other DNA
acctcaggacggactaccg

SEQ ID NO: 184 - DNA, 440 bp, synthetic construct
  source 1..440: mol_type = other DNA
acctcaggacggacttacgggataaggccggcttcatcaagagacagctggtggaaacccggcagatcacaaagcacgtggcacagatcctggactcccggatgaacactaagtacgacgagaatgacaagttgatccgggaagtgaaagtgatcaccctgaagtccaagctggtgtccgatttccggaaggatttccagttttacaaagtgcgcgagatcaacaactaccaccacgcccacgacgcctacctgaacgccgtcgtgggaaccgccctgatcaaaaagtaccctaagctggaaagcgagttcgtgtacggcgactacaaggtgtacgacgtgcggaagatgatcgccaagagcgagcaggaaatcggcaaggctaccgccaagtacttcttctacagcaacatcatgaactttttcaagaccgagataccg

SEQ ID NO: 185 - DNA, 439 bp, synthetic construct
  source 1..439: mol_type = other DNA
acctcaggacggacttacgggataaggccggcttcatcaagagacagctggtggaaacccggcagatcacaaagcacgtggcacagatcctggactcccggatgaacactaagtacgacgagaatgacaagctgatccgggaagtgaaagtgatcaccctgaagtccaagctggtgtccgatttccggaaggatttccagttttacaaagtgcgcgagatcaacaactaccaccacgcccacgacgcctacctgaacgccgtcgtgggaaccgccctgatcaaaagtaccctaagctggaaagcgagttcgtgtacggcgactacaaggtgtacgacgtgcggaagatgatcgccaagagcgagcaggaaatcggcaaggctaccgccaagtacttcttctacagcaacatcatgaactttttcaagaccgagataccg

SEQ ID NO: 186 - DNA, 20 bp, synthetic construct
  source 1..20: mol_type = other DNA
caagtgggcagcgcgccgcc

SEQ ID NO: 187 - DNA, 130 bp, Boone cardiorvirus 1
  source 1..130: mol_type = genomic DNA
ttcggttgagcccccacccggtacaacgctttaccttagaagccactaaggtgtacgcggtcatcggggacccctcctggcctttggtttattggtgaattactagttcagttaggttttgttagttagg